European Patent Application EP 4 316 597 A2, published February 7, 2024. Title: NOVEL PEPTIDES AND COMBINATION OF PEPTIDES FOR USE IN IMMUNOTHERAPY AGAINST LUNG CANCER, INCLUDING NSCLC, SCLC AND OTHER CANCERS. Applicant: immatics biotechnologies GmbH. The sequence listing filed with the application follows.

SEQUENCE LISTING (533 sequences)

SEQ ID NO: 1 - protein, 9 aa, Homo sapiens
QYDPTPLTW

SEQ ID NO: 2 - protein, 10 aa, Homo sapiens
VWSNVTPLKF

SEQ ID NO: 3 - protein, 8 aa, Homo sapiens
YLEKFYGL

SEQ ID NO: 4 - protein, 9 aa, Homo sapiens
SYEKVINYL

SEQ ID NO: 5 - protein, 9 aa, Homo sapiens
RYMKKDYLI

SEQ ID NO: 6 - protein, 9 aa, Homo sapiens
KYKDYFPVI

SEQ ID NO: 7 - protein, 9 aa, Homo sapiens
VQQWSVAVF

SEQ ID NO: 8 - protein, 10 aa, Homo sapiens
PFLPPAACFF

SEQ ID NO: 9 - protein, 9 aa, Homo sapiens
RILRFPWQL

SEQ ID NO: 10 - protein, 10 aa, Homo sapiens
VWSDVTPLNF

SEQ ID NO: 11 - protein, 11 aa, Homo sapiens
YYSKSVGFMQW

SEQ ID NO: 12 - protein, 10 aa, Homo sapiens
STIRGELFFF

SEQ ID NO: 13 - protein, 9 aa, Homo sapiens
HYTYILEVF

SEQ ID NO: 14 - protein, 8 aa, Homo sapiens
SYSSCYSF

SEQ ID NO: 15 - protein, 9 aa, Homo sapiens
KYALLLQDL

SEQ ID NO: 16 - protein, 9 aa, Homo sapiens
TYNPDFSSL

SEQ ID NO: 17 - protein, 11 aa, Homo sapiens
YYADKKTFIVL

SEQ ID NO: 18 - protein, 9 aa, Homo sapiens
DYIGSVEKW

SEQ ID NO: 19 - protein, 9 aa, Homo sapiens
ILKEDPFLF

SEQ ID NO: 20 - protein, 9 aa, Homo sapiens
EFTTVLYNF

SEQ ID NO: 21 - protein, 8 aa, Homo sapiens
SYEVRSTF

SEQ ID NO: 22 - protein, 9 aa, Homo sapiens
TQPGDWTLF

SEQ ID NO: 23 - protein, 9 aa, Homo sapiens
KFIISDWRF

SEQ ID NO: 24 - protein, 10 aa, Homo sapiens
MYPDLSELLM

SEQ ID NO: 25 - protein, 9 aa, Homo sapiens
SYNGYVFYL

SEQ ID NO: 26 - protein, 9 aa, Homo sapiens
KTPTNYYLF

SEQ ID NO: 27 - protein, 9 aa, Homo sapiens
NYTLYPITF

SEQ ID NO: 28 - protein, 9 aa, Homo sapiens
YYSIISHTL

SEQ ID NO: 29 - protein, 10 aa, Homo sapiens
VYPLLSRLYW

SEQ ID NO: 30 - protein, 10 aa, Homo sapiens
QYLPGWTVLF

SEQ ID NO: 31 - protein, 9 aa, Homo sapiens
QYQNVLTLW

SEQ ID NO: 32 - protein, 9 aa, Homo sapiens
SLPDLTPTF

SEQ ID NO: 33 - protein, 10 aa, Homo sapiens
KSSVIASLLF

SEQ ID NO: 34 - protein, 9 aa, Homo sapiens
MQPRMFFLF

SEQ ID NO: 35 - protein, 9 aa, Homo sapiens
KYLEESVWL

SEQ ID NO: 36 - protein, 10 aa, Homo sapiens
KQMEDGHTLF

SEQ ID NO: 37 - protein, 10 aa, Homo sapiens
QWPWQASLQF

SEQ ID NO: 38 - protein, 9 aa, Homo sapiens
KYTNWKAFL

SEQ ID NO: 39 - protein, 9 aa, Homo sapiens
LIFMLANVF

SEQ ID NO: 40 - protein, 12 aa, Homo sapiens
QYEPPSAPSTTF

SEQ ID NO: 41 - protein, 9 aa, Homo sapiens
VIYFMGAIF

SEQ ID NO: 42 - protein, 9 aa, Homo sapiens
TLPNTIYRF

SEQ ID NO: 43 - protein, 9 aa, Homo sapiens
IQMDEPMAF

SEQ ID NO: 44 - protein, 9 aa, Homo sapiens
AYLSAVGTF

SEQ ID NO: 45 - protein, 9 aa, Homo sapiens
KYFVPPQLF

SEQ ID NO: 46 - protein, 11 aa, Homo sapiens
AFPVTSIFHTF

SEQ ID NO: 47 - protein, 9 aa, Homo sapiens
KYADYFLEV

SEQ ID NO: 48 - protein, 11 aa, Homo sapiens
VFIDHPVHLKF

SEQ ID NO: 49 - protein, 9 aa, Homo sapiens
LYISEVRNI

SEQ ID NO: 50 - protein, 10 aa, Homo sapiens
SYPELVKMVW

SEQ ID NO: 51 - protein, 9 aa, Homo sapiens
KYALLLQEL

SEQ ID NO: 52 - protein, 9 aa, Homo sapiens
KYMKIFHKF

SEQ ID NO: 53 - protein, 9 aa, Homo sapiens
KYITNLEDL

SEQ ID NO: 54 - protein, 9 aa, Homo sapiens
LLIKLLQTF

SEQ ID NO: 55 - protein, 9 aa, Homo sapiens
RWMDQRLVF

SEQ ID NO: 56 - protein, 9 aa, Homo sapiens
VYMIEPLEL

SEQ ID NO: 57 - protein, 8 aa, Homo sapiens
YPSIIQEF

SEQ ID NO: 58 - protein, 11 aa, Homo sapiens
QFAAPLRGIYF

SEQ ID NO: 59 - protein, 9 aa, Homo sapiens
KYSTTFFMV

SEQ ID NO: 60 - protein, 9 aa, Homo sapiens
TYLSIFDQL

SEQ ID NO: 61 - protein, 9 aa, Homo sapiens
NYAENILTL

SEQ ID NO: 62 - protein, 9 aa, Homo sapiens
LYQEILAQL

SEQ ID NO: 63 - protein, 9 aa, Homo sapiens
VMPSDSFFF

SEQ ID NO: 64 - protein, 11 aa, Homo sapiens
NYAIFDEGHML

SEQ ID NO: 65 - protein, 11 aa, Homo sapiens
VYPASKMFPFI

SEQ ID NO: 66 - protein, 9 aa, Homo sapiens
IYFRDSSFL

SEQ ID NO: 67 - protein, 9 aa, Homo sapiens
RYPGKFYRV

SEQ ID NO: 68 - protein, 9 aa, Homo sapiens
IYQQIIQTY

SEQ ID NO: 69 - protein, 9 aa, Homo sapiens
IMPEKFEFW

SEQ ID NO: 70 - protein, 9 aa, Homo sapiens
PYTNYTFDF

SEQ ID NO: 71 - protein, 9 aa, Homo sapiens
SYMVLAPVF

SEQ ID NO: 72 - protein, 9 aa, Homo sapiens
RYEGILYTI

SEQ ID NO: 73 - protein, 9 aa, Homo sapiens
SYIGLPLTL

SEQ ID NO: 74 - protein, 9 aa, Homo sapiens
VYDQYFITL

SEQ ID NO: 75 - protein, 9 aa, Homo sapiens
NYIYSISVF

SEQ ID NO: 76 - protein, 9 aa, Homo sapiens
WYGWHFPEL

SEQ ID NO: 77 - protein, 10 aa, Homo sapiens
AYTLLGHEFV

SEQ ID NO: 78 - protein, 10 aa, Homo sapiens
TWFPKTPMLF

SEQ ID NO: 79 - protein, 9 aa, Homo sapiens
RYLADLPTL

SEQ ID NO: 80 - protein, 9 aa, Homo sapiens
YYSPLRDLL

SEQ ID NO: 81 - protein, 9 aa, Homo sapiens
LYPEGLRLL

SEQ ID NO: 82 - protein, 9 aa, Homo sapiens
RFLPSPVVI

SEQ ID NO: 83 - protein, 9 aa, Homo sapiens
TYCQNIKEF

SEQ ID NO: 84 - protein, 9 aa, Homo sapiens
YVDINTFRL

SEQ ID NO: 85 - protein, 9 aa, Homo sapiens
YIDEFQSLV

SEQ ID NO: 86 - protein, 9 aa, Homo sapiens
FVIDGFDEL

SEQ ID NO: 87 - protein, 10 aa, Homo sapiens
TLYPYQISQL

SEQ ID NO: 88 - protein, 11 aa, Homo sapiens
VQMVITEAQKV

SEQ ID NO: 89 - protein, 9 aa, Homo sapiens
ILSTTMVTV

SEQ ID NO: 90 - protein, 8 aa, Homo sapiens
FLLMHPSI

SEQ ID NO: 91 - protein, 9 aa, Homo sapiens
FALPGLLHA

SEQ ID NO: 92 - protein, 9 aa, Homo sapiens
NLRDLLSEV

SEQ ID NO: 93 - protein, 9 aa, Homo sapiens
TLQEKILQV

SEQ ID NO: 94 - protein, 11 aa, Homo sapiens
VLPDIETLIGV

SEQ ID NO: 95 - protein, 9 aa, Homo sapiens
ITIGVLARV

SEQ ID NO: 96 - protein, 9 aa, Homo sapiens
HLVGGLHTV

SEQ ID NO: 97 - protein, 9 aa, Homo sapiens
VLALVNSTV

SEQ ID NO: 98 - protein, 10 aa, Homo sapiens
LQSSGLTLLL

SEQ ID NO: 99 - protein, 9 aa, Homo sapiens
FLKEKVPGI

SEQ ID NO: 100 - protein, 9 aa, Homo sapiens
RQYPTPFQL

SEQ ID NO: 101 - protein, 10 aa, Homo sapiens
FIISDWRFVL

SEQ ID NO: 102 - protein, 9 aa, Homo sapiens
SLLEQAIAL

SEQ ID NO: 103 - protein, 9 aa, Homo sapiens
FLYYPDPVL

SEQ ID NO: 104 - protein, 9 aa, Homo sapiens
GMLDIFWGV

SEQ ID NO: 105 - protein, 9 aa, Homo sapiens
SLLTHIPTA

SEQ ID NO: 106 - protein, 11 aa, Homo sapiens
FIIDTTYPAYV

SEQ ID NO: 107 - protein, 9 aa, Homo sapiens
LLQGAIESV

SEQ ID NO: 108 - protein, 9 aa, Homo sapiens
MIIALSLYI

SEQ ID NO: 109 - protein, 11 aa, Homo sapiens
LLLGSIGLLGV

SEQ ID NO: 110 - protein, 9 aa, Homo sapiens
LLADFQALL

SEQ ID NO: 111 - protein, 9 aa, Homo sapiens
ALCLLLHLL

SEQ ID NO: 112 - protein, 9 aa, Homo sapiens
SVSDGIHSV

SEQ ID NO: 113 - protein, 9 aa, Homo sapiens
AVLTGLVEV

SEQ ID NO: 114 - protein, 9 aa, Homo sapiens
ILDERQVLL

SEQ ID NO: 115 - protein, 11 aa, Homo sapiens
MLLETQDALYV

SEQ ID NO: 116 - protein, 9 aa, Homo sapiens
VLMEENSKL

SEQ ID NO: 117 - protein, 10 aa, Homo sapiens
FLDPNARPLV

SEQ ID NO: 118 - protein, 9 aa, Homo sapiens
ALSSVLHSI

SEQ ID NO: 119 - protein, 9 aa, Homo sapiens
RTADITVTV

SEQ ID NO: 120 - protein, 9 aa, Homo sapiens
ALLANLPAV

SEQ ID NO: 121 - protein, 9 aa, Homo sapiens
ALVDTLTGI

SEQ ID NO: 122 - protein, 11 aa, Homo sapiens
ALLEMFPEITV

SEQ ID NO: 123 - protein, 9 aa, Homo sapiens
LMAFFLAVV

SEQ ID NO: 124 - protein, 9 aa, Homo sapiens
SVASVLLYL

SEQ ID NO: 125 - protein, 9 aa, Homo sapiens
VLQPFLPSI

SEQ ID NO: 126 - protein, 8 aa, Homo sapiens
FLSTVTSV

SEQ ID NO: 127 - protein, 9 aa, Homo sapiens
GLDGSLVFL

SEQ ID NO: 128 - protein, 8 aa, Homo sapiens
FLGTTPTL

SEQ ID NO: 129 - protein, 10 aa, Homo sapiens
VLYDKDAVYV

SEQ ID NO: 130 - protein, 11 aa, Homo sapiens
NLWGGQGLLGV

SEQ ID NO: 131 - protein, 9 aa, Homo sapiens
LLKEFVQRV

SEQ ID NO: 132 - protein, 10 aa, Homo sapiens
ALWLVDPLTV

SEQ ID NO: 133 - protein, 11 aa, Homo sapiens
MTLPVDAVISV

SEQ ID NO: 134 - protein, 11 aa, Homo sapiens
AAEIGDKSWLY

SEQ ID NO: 135 - protein, 9 aa, Homo sapiens
ASEDSVLLY

SEQ ID NO: 136 - protein, 10 aa, Homo sapiens
ATDLVVLDRY

SEQ ID NO: 137 - protein, 9 aa, Homo sapiens
ATSKFMEFY

SEQ ID NO: 138 - protein, 9 aa, Homo sapiens
DSDSCHFNY

SEQ ID NO: 139 - protein, 9 aa, Homo sapiens
ECDMAFHIY

SEQ ID NO: 140 - protein, 9 aa, Homo sapiens
ESDREELNY

SEQ ID NO: 141 - protein, 9 aa, Homo sapiens
ESDVGVVVY

SEQ ID NO: 142 - protein, 12 aa, Homo sapiens
EVAEPSVLFDLY

SEQ ID NO: 143 - protein, 10 aa, Homo sapiens
FIDYPKKEDY

SEQ ID NO: 144 - protein, 10 aa, Homo sapiens
FLDSQNLSAY

SEQ ID NO: 145 - protein, 8 aa, Homo sapiens
FVDKPVAY

SEQ ID NO: 146 - protein, 10 aa, Homo sapiens
GLNTGSALSY

SEQ ID NO: 147 - protein, 11 aa, Homo sapiens
GSSDSSTLPKL

SEQ ID NO: 148 - protein, 9 aa, Homo sapiens
GTEFTTILY

SEQ ID NO: 149 - protein, 9 aa, Homo sapiens
GTEFTTVLY

SEQ ID NO: 150 - protein, 9 aa, Homo sapiens
GTELLSLVY

SEQ ID NO: 151 - protein, 9 aa, Homo sapiens
HSDLKVGEY

SEQ ID NO: 152 - protein, 9 aa, Homo sapiens
HTDSLHLLI

SEQ ID NO: 153 - protein, 10 aa, Homo sapiens
KLDRSVFTAY

SEQ ID NO: 154 - protein, 10 aa, Homo sapiens
LLDISQKNLY

SEQ ID NO: 155 - protein, 9 aa, Homo sapiens
LLDPNPHMY

SEQ ID NO: 156 - protein, 9 aa, Homo sapiens
LLDSLREQY

SEQ ID NO: 157 - protein, 8 aa, Homo sapiens
LMDRPIFY

SEQ ID NO: 158 - protein, 9 aa, Homo sapiens
LSDLLKQGY

SEQ ID NO: 159 - protein, 10 aa, Homo sapiens
LSDTSVIQFY

SEQ ID NO: 160 - protein, 9 aa, Homo sapiens
LTEAVLNRY

SEQ ID NO: 161 - protein, 10 aa, Homo sapiens
LVDDGTHGQY

SEQ ID NO: 162 - protein, 11 aa, Homo sapiens
LVDNSIRELQY

SEQ ID NO: 163 - protein, 12 aa, Homo sapiens
NSDSSLTLREFY

SEQ ID NO: 164 - protein, 9 aa, Homo sapiens
NTDNNLAVY

SEQ ID NO: 165 - protein, 9 aa, Homo sapiens
NTDPTAPPY

SEQ ID NO: 166 - protein, 10 aa, Homo sapiens
NTQITDIGRY

SEQ ID NO: 167 - protein, 11 aa, Homo sapiens
QSDPGTSVLGY

SEQ ID NO: 168 - protein, 12 aa, Homo sapiens
QTDHPQPILDRY

SEQ ID NO: 169 - protein, 10 aa, Homo sapiens
RLDTPLYFSY

SEQ ID NO: 170 - protein, 9 aa, Homo sapiens
RSDDTAVYY

SEQ ID NO: 171 - protein, 11 aa, Homo sapiens
RSDPVTLNVLY

SEQ ID NO: 172 - protein, 12 aa, Homo sapiens
RTDSCSSAQAQY

SEQ ID NO: 173 - protein, 9 aa, Homo sapiens
RTEFNLNQY

SEQ ID NO: 174 - protein, 12 aa, Homo sapiens
SADDIRGIQSLY

SEQ ID NO: 175 - protein, 8 aa, Homo sapiens
SDVTPLTF

SEQ ID NO: 176 - protein, 10 aa, Homo sapiens
SRTINVSNLY

SEQ ID NO: 177 - protein, 10 aa, Homo sapiens
SSDEVNFLVY

SEQ ID NO: 178 - protein, 10 aa, Homo sapiens
SSDSSTLPKL

SEQ ID NO: 179 - protein, 10 aa, Homo sapiens
STAKSATWTY

SEQ ID NO: 180 - protein, 10 aa, Homo sapiens
STDPWIQMAY

SEQ ID NO: 181 - protein, 9 aa, Homo sapiens
TADGKTYYY

SEQ ID NO: 182 - protein, 8 aa, Homo sapiens
TDYHVRVY

SEQ ID NO: 183 - protein, 11 aa, Homo sapiens
TLEDIATSHLY

SEQ ID NO: 184 - protein, 11 aa, Homo sapiens
TSAHPEDSSFY

SEQ ID NO: 185 - protein, 9 aa, Homo sapiens
TSDSNLNKY

SEQ ID NO: 186 - protein, 8 aa, Homo sapiens
TTDIIEKY

SEQ ID NO: 187 - protein, 9 aa, Homo sapiens
VADLHLYLY

SEQ ID NO: 188 - protein, 9 aa, Homo sapiens
VSDAKLDKY

SEQ ID NO: 189 - protein, 10 aa, Homo sapiens
VSDSECLSRY

SEQ ID NO: 190 - protein, 12 aa, Homo sapiens
VTDGINPLIDRY

SEQ ID NO: 191 - protein, 12 aa, Homo sapiens
VTDGSLYEGVAY

SEQ ID NO: 192 - protein, 11 aa, Homo sapiens
VTEESFDSKFY

SEQ ID NO: 193 - protein, 9 aa, Homo sapiens
VTEFSLNTY

SEQ ID NO: 194 - protein, 10 aa, Homo sapiens
VVADTKMIEY

SEQ ID NO: 195 - protein, 10 aa, Homo sapiens
VVDSVGGYLY

SEQ ID NO: 196 - protein, 8 aa, Homo sapiens
WMFFVINY

SEQ ID NO: 197 - protein, 10 aa, Homo sapiens
YADTVRPEFY

SEQ ID NO: 198 - protein, 10 aa, Homo sapiens
YLDPVQRDLY

SEQ ID NO: 199 - protein, 10 aa, Homo sapiens
YLPQHTIETY

SEQ ID NO: 200 - protein, 9 aa, Homo sapiens
YSDEDVTKY

SEQ ID NO: 201 - protein, 9 aa, Homo sapiens
YVGKEHMFY

SEQ ID NO: 202 - protein, 11 aa, Homo sapiens
KLAELEGALQK

SEQ ID NO: 203 - protein, 10 aa, Homo sapiens
KVKDTPGLGK

SEQ ID NO: 204 - protein, 9 aa, Homo sapiens
AVFDKFIRY

SEQ ID NO: 205 - protein, 9 aa, Homo sapiens
SLDGAARPK

SEQ ID NO: 206 - protein, 10 aa, Homo sapiens
KLIDLSQVMY

SEQ ID NO: 207 - protein, 10 aa, Homo sapiens
RSFNGLLTMY

SEQ ID NO: 208 - protein, 10 aa, Homo sapiens
GLASRILDAK

SEQ ID NO: 209 - protein, 9 aa, Homo sapiens
RTQIPMSEK

SEQ ID NO: 210 - protein, 9 aa, Homo sapiens
ATSGVPVYK

SEQ ID NO: 211 - protein, 9 aa, Homo sapiens
TVNPVAIHK

SEQ ID NO: 212 - protein, 9 aa, Homo sapiens
KAYEQVMHY

SEQ ID NO: 213 - protein, 12 aa, Homo sapiens
LNINMTSPMGTK

SEQ ID NO: 214 - protein, 11 aa, Homo sapiens
RTMSEAALVRK

SEQ ID NO: 215 - protein, 11 aa, Homo sapiens
MMFSGPQILKL

SEQ ID NO: 216 - protein, 9 aa, Homo sapiens
KLYAWELAF

SEQ ID NO: 217 - protein, 9 aa, Homo sapiens
RILNQILYY

SEQ ID NO: 218 - protein, 11 aa, Homo sapiens
KTLVAELLILK

SEQ ID NO: 219 - protein, 9 aa, Homo sapiens
RLRSSLVFK

SEQ ID NO: 220 - protein, 10 aa, Homo sapiens
SPSVSQLSVL

SEQ ID NO: 221 - protein, 9 aa, Homo sapiens
VPDVAQFVL

SEQ ID NO: 222 - protein, 9 aa, Homo sapiens
NPFYPEVEL

SEQ ID NO: 223 - protein, 9 aa, Homo sapiens
YPKDIYSSF

SEQ ID NO: 224 - protein, 9 aa, Homo sapiens
GPQPWHAAL

SEQ ID NO: 225 - protein, 10 aa, Homo sapiens
LPFDGPGGIL

SEQ ID NO: 226 - protein, 11 aa, Homo sapiens
SPRMSGLLSQT

SEQ ID NO: 227 - protein, 11 aa, Homo sapiens
YPRGNHWAVGH

SEQ ID NO: 228 - protein, 12 aa, Homo sapiens
YPRGNHWAVGHL

SEQ ID NO: 229 - protein, 10 aa, Homo sapiens
VPLPAGGGTV

SEQ ID NO: 230 - protein, 11 aa, Homo sapiens
VPLPAGGGTVL

SEQ ID NO: 231 - protein, 10 aa, Homo sapiens
RPRALRDLQL

SEQ ID NO: 232 - protein, 11 aa, Homo sapiens
RPRALRDLQLL

SEQ ID NO: 233 - protein, 9 aa, Homo sapiens
KPYQGNPTF

SEQ ID NO: 234 - protein, 9 aa, Homo sapiens
RAKNAGVTI

SEQ ID NO: 235 - protein, 9 aa, Homo sapiens
MPLKHYLLL

SEQ ID NO: 236 - protein, 12 aa, Homo sapiens
RVRGGEDGDRAL

SEQ ID NO: 237 - protein, 10 aa, Homo sapiens
RPAATAVISL

SEQ ID NO: 238 - protein, 9 aa, Homo sapiens
KPGPPWAAF

SEQ ID NO: 239 - protein, 10 aa, Homo sapiens
YVPSASLFML

SEQ ID NO: 240 - protein, 9 aa, Homo sapiens
SPREVTTVL

SEQ ID NO: 241 - protein, 9 aa, Homo sapiens
SARLATDAL

SEQ ID NO: 242 - protein, 9 aa, Homo sapiens
SPRWLPVSL

SEQ ID NO: 243 - protein, 10 aa, Homo sapiens
RPIENRILIL

SEQ ID NO: 244 - protein, 9 aa, Homo sapiens
FPYVRDFVM

SEQ ID NO: 245 - protein, 9 aa, Homo sapiens
RIREHVPQL

SEQ ID NO: 246 - protein, 9 aa, Homo sapiens
TPLPAVIVL

SEQ ID NO: 247 - protein, 9 aa, Homo sapiens
RALLARLLL

SEQ ID NO: 248 - protein, 9 aa, Homo sapiens
IPNWARQDL

SEQ ID NO: 249 - protein, 9 aa, Homo sapiens
VPSSRILQL

SEQ ID NO: 250 - protein, 9 aa, Homo sapiens
SPRDFLSGL

SEQ ID NO: 251 - protein, 9 aa, Homo sapiens
VPRSSGQTV

SEQ ID NO: 252 - protein, 9 aa, Homo sapiens
SPDIRNTTV

SEQ ID NO: 253 - protein, 10 aa, Homo sapiens
RVIDAVRFTL

SEQ ID NO: 254 - protein, 9 aa, Homo sapiens
NPFPHLITL

SEQ ID NO: 255 - protein, 9 aa, Homo sapiens
MPLLENLYL

SEQ ID NO: 256 - protein, 9 aa, Homo sapiens
SPRVPSIEL

SEQ ID NO: 257 - protein, 9 aa, Homo sapiens
LPRIPFADV

SEQ ID NO: 258 - protein, 9 aa, Homo sapiens
LPRGPLASL

SEQ ID NO: 259 - protein, 12 aa, Homo sapiens
RPPAAGLRGISL

SEQ ID NO: 260 - protein, 9 aa, Homo sapiens
YPQHPGLNA

SEQ ID NO: 261 - protein, 9 aa, Homo sapiens
APSARVGVC

SEQ ID NO: 262 - protein, 9 aa, Homo sapiens
SAYPQRLEI

SEQ ID NO: 263 - protein, 9 aa, Homo sapiens
HPAPYGDLL

SEQ ID NO: 264 - protein, 9 aa, Homo sapiens
RPILIIITL

SEQ ID NO: 265 - protein, 9 aa, Homo sapiens
SPRQPPRLV

SEQ ID NO: 266 - protein, 9 aa, Homo sapiens
HAYPPGPGL

SEQ ID NO: 267 - protein, 10 aa, Homo sapiens
HPELVNHIVF

SEQ ID NO: 268 - protein, 9 aa, Homo sapiens
YPLFRGINL

SEQ ID NO: 269 - protein, 9 aa, Homo sapiens
APRAPRLML

SEQ ID NO: 270 - protein, 9 aa, Homo sapiens
APGPRFLVT

SEQ ID NO: 271 - protein, 10 aa, Homo sapiens
MPLPWSLALP

SEQ ID NO: 272 - protein, 11 aa, Homo sapiens
MPLPWSLALPL

SEQ ID NO: 273 - protein, 9 aa, Homo sapiens
MPLLWLRGF

SEQ ID NO: 274 - protein, 9 aa, Homo sapiens
TPYQEHVAL

SEQ ID NO: 275 - protein, 9 aa, Homo sapiens
APHPPLSVV

SEQ ID NO: 276 - protein, 9 aa, Homo sapiens
LPRAGGAFL

SEQ ID NO: 277 - protein, 9 aa, Homo sapiens
MPLFEPRVF

SEQ ID NO: 278 - protein, 12 aa, Homo sapiens
HPMIDINGIIVF

SEQ ID NO: 279 - protein, 9 aa, Homo sapiens
SPARASPAL

SEQ ID NO: 280 - protein, 11 aa, Homo sapiens
VPISEEGTPVL

SEQ ID NO: 281 - protein, 9 aa, Homo sapiens
RPRAPVTPA

SEQ ID NO: 282 - protein, 10 aa, Homo sapiens
MPQIETRVIL

SEQ ID NO: 283 - protein, 9 aa, Homo sapiens
RPHSLSSEL

SEQ ID NO: 284 - protein, 10 aa, Homo sapiens
FPVTSIFHTF

SEQ ID NO: 285 - protein, 9 aa, Homo sapiens
FPSFLTNSL

SEQ ID NO: 286 - protein, 8 aa, Homo sapiens
VPTLRSEL

SEQ ID NO: 287 - protein, 10 aa, Homo sapiens
APREEQQRSL

SEQ ID NO: 288 - protein, 9 aa, Homo sapiens
FPQKFIDLL

SEQ ID NO: 289 - protein, 9 aa, Homo sapiens
VPENHSVAL

SEQ ID NO: 290 - protein, 10 aa, Homo sapiens
APYRPPDISL

SEQ ID NO: 291 - protein, 9 aa, Homo sapiens
SPQRLRGLL

SEQ ID NO: 292 - protein, 10 aa, Homo sapiens
SPQRLRGLLL

SEQ ID NO: 293 - protein, 12 aa, Homo sapiens
RPRSALPRLLLP

SEQ ID NO: 294 - protein, 10 aa, Homo sapiens
GPTPNTGAAL

SEQ ID NO: 295 - protein, 9 aa, Homo sapiens
KPEGTRIAV

SEQ ID NO: 296 - protein, 8 aa, Homo sapiens
MPMQDIKM

SEQ ID NO: 297 - protein, 9 aa, Homo sapiens
RAQLKLVAL

SEQ ID NO: 298 - protein, 9 aa, Homo sapiens
FNKRKPLSL

SEQ ID NO: 299 - protein, 9 aa, Homo sapiens
MAQFKEISL

SEQ ID NO: 300 - protein, 9 aa, Homo sapiens
VASPKHCVL

SEQ ID NO: 301 - protein, 8 aa, Homo sapiens
YMHKLLVL

SEQ ID NO: 302 - protein, 9 aa, Homo sapiens
HLLQKQTSI

SEQ ID NO: 303 - protein, 8 aa, Homo sapiens
LPFPKFTV

SEQ ID NO: 304 - protein, 9 aa, Homo sapiens
ELKKLYCQI

SEQ ID NO: 305 - protein, 9 aa, Homo sapiens
ALKLRVAVL

SEQ ID NO: 306 - protein, 8 aa, Homo sapiens
ILKVKVGL

SEQ ID NO: 307 - protein, 9 aa, Homo sapiens
ILLPRTVSL

SEQ ID NO: 308 - protein, 9 aa, Homo sapiens
MLKQKVEEL

SEQ ID NO: 309 - protein, 9 aa, Homo sapiens
DAIQRKYSC

SEQ ID NO: 310 - protein, 8 aa, Homo sapiens
LPPKKFVL

SEQ ID NO: 311 - protein, 9 aa, Homo sapiens
EIRIRVVQM

SEQ ID NO: 312 - protein, 9 aa, Homo sapiens
EAMLRNKEL

SEQ ID NO: 313 - protein, 10 aa, Homo sapiens
ELKKKEYEEL

SEQ ID NO: 314 - protein, 9 aa, Homo sapiens
AIISRLVAL

SEQ ID NO: 315 - protein, 9 aa, Homo sapiens
DIYQRALNL

SEQ ID NO: 316 - protein, 9 aa, Homo sapiens
VIKEKALTL

SEQ ID NO: 317 - protein, 8 aa, Homo sapiens
LVKVKVLL

SEQ ID NO: 318 - protein, 9 aa, Homo sapiens
EAAIRSVEL

SEQ ID NO: 319 - protein, 11 aa, Homo sapiens
AEMLERVIKNY

SEQ ID NO: 320 - protein, 12 aa, Homo sapiens
MEVDPIGHVYIF

SEQ ID NO: 321 - protein, 11 aa, Homo sapiens
AEMLESVIKNY

SEQ ID NO: 322 - protein, 10 aa, Homo sapiens
KEVDPAGHSY

SEQ ID NO: 323 - protein, 8 aa, Homo sapiens
SEFMQVIF

SEQ ID NO: 324 - protein, 9 aa, Homo sapiens
TDSIHAWTF

SEQ ID NO: 325 - protein, 11 aa, Homo sapiens
QEQDVDLVQKY

SEQ ID NO: 326 - protein, 9 aa, Homo sapiens
QEMQHFLGL

SEQ ID NO: 327 - protein, 10 aa, Homo sapiens
YEIEARNQVF

SEQ ID NO: 328 - protein, 10 aa, Homo sapiens
FEYDFLLQRI

SEQ ID NO: 329 - protein, 8 aa, Homo sapiens
NEHPSNNW

SEQ ID NO: 330 - protein, 10 aa, Homo sapiens
KEGDLGGKQW

SEQ ID NO: 331 - protein, 8 aa, Homo sapiens
EDAQGHIW

SEQ ID NO: 332 - protein, 8 aa, Homo sapiens
MEVPVIKI

SEQ ID NO: 333 - protein, 9 aa, Homo sapiens
AETLSTIQI

SEQ ID NO: 334 - protein, 10 aa, Homo sapiens
AEDEPAAAHL

SEQ ID NO: 335 - protein, 9 aa, Homo sapiens
KELEATKQY

SEQ ID NO: 336 - protein, 10 aa, Homo sapiens
ASSSGPMRWW

SEQ ID NO: 337 - protein, 9 aa, Homo sapiens
TENRYCVQL

SEQ ID NO: 338 - protein, 12 aa, Homo sapiens
SEGSEPALLHSW

SEQ ID NO: 339 - protein, 9 aa, Homo sapiens
SEPALLHSW

SEQ ID NO: 340 - protein, 8 aa, Homo sapiens
TEFSLNTY

SEQ ID NO: 341 - protein, 12 aa, Homo sapiens
EEIEGKGSFTYF

SEQ ID NO: 342 - protein, 9 aa, Homo sapiens
HEFSSPSHL

SEQ ID NO: 343 - protein, 8 aa, Homo sapiens
TEFTTVLY

SEQ ID NO: 344 - protein, 10 aa, Homo sapiens
EEATGQFHVY

SEQ ID NO: 345 - protein, 9 aa, Homo sapiens
IEFIHPQAF

SEQ ID NO: 346 - protein, 11 aa, Homo sapiens
VEAPGPVHVYW

SEQ ID NO: 347 - protein, 9 aa, Homo sapiens
ALNPYQYQY

SEQ ID NO: 348 - protein, 10 aa, Homo sapiens
AEIQGNINHV

SEQ ID NO: 349 - protein, 10 aa, Homo sapiens
AEQDMRELTY

SEQ ID NO: 350 - protein, 10 aa, Homo sapiens
GECDVFKEIL

SEQ ID NO: 351 - protein, 9 aa, Homo sapiens
EEVNYINTF

SEQ ID NO: 352 - protein, 9 aa, Homo sapiens
NEVLTYIKF

SEQ ID NO: 353 - protein, 9 aa, Homo sapiens
GEIIMQNNW

SEQ ID NO: 354 - protein, 9 aa, Homo sapiens
TEDPTILRI

SEQ ID NO: 355 - protein, 9 aa, Homo sapiens
SDMVRFHLF

SEQ ID NO: 356 - protein, 8 aa, Homo sapiens
EEGRVYLF

SEQ ID NO: 357 - protein, 10 aa, Homo sapiens
RELENCFQIQ

SEQ ID NO: 358 - protein, 9 aa, Homo sapiens
KEADIHFLI

SEQ ID NO: 359 - protein, 9 aa, Homo sapiens
DELFSIALY

SEQ ID NO: 360 - protein, 9 aa, Homo sapiens
AEVPTGVII

SEQ ID NO: 361 - protein, 9 aa, Homo sapiens
SENLFFASF

SEQ ID NO: 362 - protein, 9 aa, Homo sapiens
SEKGVIQVY

SEQ ID NO: 363 - protein, 9 aa, Homo sapiens
AELDKLTSV

SEQ ID NO: 364 - protein, 9 aa, Homo sapiens
AETPIQNVI

SEQ ID NO: 365 - protein, 9 aa, Homo sapiens
SEMNVNMKY

SEQ ID NO: 366 - protein, 8 aa, Homo sapiens
AENLFRAF

SEQ ID NO: 367 - protein, 9 aa, Homo sapiens
GEVHPSEMI

SEQ ID NO: 368 - protein, 9 aa, Homo sapiens
GEFPVRVQV

SEQ ID NO: 369 - protein, 9 aa, Homo sapiens
EEIERFFKL

SEQ ID NO: 370 - protein, 8 aa, Homo sapiens
YEDLSQKY

SEQ ID NO: 371 - protein, 9 aa, Homo sapiens
GELALKKKI

SEQ ID NO: 372 - protein, 9 aa, Homo sapiens
TEGIIMKDF

SEQ ID NO: 373 - protein, 9 aa, Homo sapiens
MEMQKSPVF

SEQ ID NO: 374 - protein, 8 aa, Homo sapiens
DEVNFLVY

SEQ ID NO: 375 - protein, 10 aa, Homo sapiens
VYSDLHAFYY

SEQ ID NO: 376 - protein, 9 aa, Homo sapiens
KYVKDFHKF

SEQ ID NO: 377 - protein, 9 aa, Homo sapiens
VYVGAVNRI

SEQ ID NO: 378 - protein, 11 aa, Homo sapiens
KFLGPAEHLTF

SEQ ID NO: 379 - protein, 10 aa, Homo sapiens
NYIVPDKQIF

SEQ ID NO: 380 - protein, 9 aa, Homo sapiens
VFQEKHHVI

SEQ ID NO: 381 - protein, 9 aa, Homo sapiens
TYSKKHFRI

SEQ ID NO: 382 - protein, 9 aa, Homo sapiens
IYHSHHPTL

SEQ ID NO: 383 - protein, 9 aa, Homo sapiens
RYKQDVERF

SEQ ID NO: 384 - protein, 9 aa, Homo sapiens
KYVKVFDKF

SEQ ID NO: 385 - protein, 9 aa, Homo sapiens
MYINEVERL

SEQ ID NO: 386 - protein, 10 aa, Homo sapiens
VYNDHSIYVW

SEQ ID NO: 387 - protein, 11 aa, Homo sapiens
RWLPQKNAAQF

SEQ ID NO: 388 - protein, 11 aa, Homo sapiens
FSIPEGALVAV

SEQ ID NO: 389 - protein, 10 aa, Homo sapiens
TLMEQPLTTL

SEQ ID NO: 390 - protein, 9 aa, Homo sapiens
HIMPTVHTV

SEQ ID NO: 391 - protein, 11 aa, Homo sapiens
SLIDMRGIETV

SEQ ID NO: 392 - protein, 9 aa, Homo sapiens
SLFKDQMEL

SEQ ID NO: 393 - protein, 9 aa, Homo sapiens
ILLPYLQTL

SEQ ID NO: 394 - protein, 10 aa, Homo sapiens
ASEAEMRLFY

SEQ ID NO: 395 - protein, 10 aa, Homo sapiens
ASEASRLAHY

SEQ ID NO: 396 - protein, 10 aa, Homo sapiens
ASEFGNHYLY

SEQ ID NO: 397 - protein, 12 aa, Homo sapiens
ASEITSKGASLY

SEQ ID NO: 398 - protein, 12 aa, Homo sapiens
ASEQQALHTVQY

SEQ ID NO: 399 - protein, 9 aa, Homo sapiens
ATDIPCLLY

SEQ ID NO: 400 - protein, 10 aa, Homo sapiens
ATDISRQNEY

SEQ ID NO: 401 - protein, 12 aa, Homo sapiens
DSDESYMEKSLY

SEQ ID NO: 402 - protein, 9 aa, Homo sapiens
DTDSQRLAY

SEQ ID NO: 403 - protein, 11 aa, Homo sapiens
ELDSKVEVLTY

SEQ ID NO: 404 - protein, 9 aa, Homo sapiens
ETARKFLYY

SEQ ID NO: 405 - protein, 10 aa, Homo sapiens
ETEEGIYWRY

SEQ ID NO: 406 - protein, 10 aa, Homo sapiens
ETEQTKFWDY

SEQ ID NO: 407 - protein, 10 aa, Homo sapiens
FSDNDKLYLY

SEQ ID NO: 408 - protein, 9 aa, Homo sapiens
FTEQWTDGY

SEQ ID NO: 409 - protein, 9 aa, Homo sapiens
FVDPLVTNY

SEQ ID NO: 410 - protein, 12 aa, Homo sapiens
GSDHQSPSSSSY

SEQ ID NO: 411 - protein, 9 aa, Homo sapiens
GTVYEDLRY

SEQ ID NO: 412 - protein, 9 aa, Homo sapiens
ILDEVIMGY

SEQ ID NO: 413 - protein, 10 aa, Homo sapiens
ISDRYYTALY

SEQ ID NO: 414 - protein, 9 aa, Homo sapiens
KTDESLTKY

SEQ ID NO: 415 - protein, 10 aa, Homo sapiens
LLDPRSYHTY

SEQ ID NO: 416 - protein, 10 aa, Homo sapiens
LLDTAQKNLY

SEQ ID NO: 417 - protein, 10 aa, Homo sapiens
LLEDKHFQSY

SEQ ID NO: 418 - protein, 10 aa, Homo sapiens
LSDPSGPKSY

SEQ ID NO: 419 - protein, 9 aa, Homo sapiens
LSELKPMSY

SEQ ID NO: 420 - protein, 10 aa, Homo sapiens
LTEDKETLQY

SEQ ID NO: 421 - protein, 11 aa, Homo sapiens
LTELLERAAFY

SEQ ID NO: 422 - protein, 9 aa, Homo sapiens
MIDVTKSYY

SEQ ID NO: 423 - protein, 12 aa, Homo sapiens
NLDAVHDITVAY

SEQ ID NO: 424 - protein, 10 aa, Homo sapiens
NLDEEKQLLY

SEQ ID NO: 425 - protein, 9 aa, Homo sapiens
NLDIIQQEY

SEQ ID NO: 426 - protein, 10 aa, Homo sapiens
NLDQATRVAY

SEQ ID NO: 427 - protein, 12 aa, Homo sapiens
NSDEQKITEMVY

SEQ ID NO: 428 - protein, 9 aa, Homo sapiens
NSELSCQLY

SEQ ID NO: 429 - protein, 12 aa, Homo sapiens
NTEDSSMSGYLY

SEQ ID NO: 430 - protein, 9 aa, Homo sapiens
NTEGLHHLY

SEQ ID NO: 431 - protein, 11 aa, Homo sapiens
NTSDMMGRMSY

SEQ ID NO: 432 - protein, 9 aa, Homo sapiens
NVDPVQHTY

SEQ ID NO: 433 - protein, 9 aa, Homo sapiens
QIDTGENLY

SEQ ID NO: 434 - protein, 10 aa, Homo sapiens
QTDCAPNNGY

SEQ ID NO: 435 - protein, 10 aa, Homo sapiens
QTDDTWRTEY

SEQ ID NO: 436 - protein, 11 aa, Homo sapiens
QTETGTPYMLY

SEQ ID NO: 437 - protein, 10 aa, Homo sapiens
STDGKHWWEY

SEQ ID NO: 438 - protein, 9 aa, Homo sapiens
STDNFNCKY

SEQ ID NO: 439 - protein, 10 aa, Homo sapiens
TLDAGKFQIY

SEQ ID NO: 440 - protein, 10 aa, Homo sapiens
TLDENPGVRY

SEQ ID NO: 441 - protein, 12 aa, Homo sapiens
TLDSALNAASYY

SEQ ID NO: 442 - protein, 10 aa, Homo sapiens
TSDFSRFTNY

SEQ ID NO: 443 - protein, 12 aa, Homo sapiens
TTDFPSESSFEY

SEQ ID NO: 444 - protein, 9 aa, Homo sapiens
TTDTVIRSY

SEQ ID NO: 445 - protein, 10 aa, Homo sapiens
VLDQGKITEY

SEQ ID NO: 446 - protein, 11 aa, Homo sapiens
VTAQVVGTERY

SEQ ID NO: 447 - protein, 10 aa, Homo sapiens
VVDEDHELIY

SEQ ID NO: 448 - protein, 9 aa, Homo sapiens
YLDIPNPRY

SEQ ID NO: 449 - protein, 12 aa, Homo sapiens
YLDRGTGNVSFY

SEQ ID NO: 450 - protein, 11 aa, Homo sapiens
YSDDGQKWTVY

SEQ ID NO: 451 - protein, 10 aa, Homo sapiens
YSDSLVQKGY

SEQ ID NO: 452 - protein, 12 aa, Homo sapiens
YVDAVLGKGHQY

SEQ ID NO: 453 - protein, 9 aa, Homo sapiens
AINTSIKNK

SEQ ID NO: 454 - protein, 9 aa, Homo sapiens
KVYTPSISK

SEQ ID NO: 455 - protein, 9 aa, Homo sapiens
RIADIFVKK

SEQ ID NO: 456 - protein, 9 aa, Homo sapiens
SMFTAILKK

SEQ ID NO: 457 - protein, 9 aa, Homo sapiens
SINKPTSER

SEQ ID NO: 458 - protein, 9 aa, Homo sapiens
GIADFVLKY

SEQ ID NO: 459 - protein, 10 aa, Homo sapiens
RPMQQARAQL

SEQ ID NO: 460 - protein, 10 aa, Homo sapiens
MPMAGDMNGL

SEQ ID NO: 461 - protein, 9 aa, Homo sapiens
RPILIIVTL

SEQ ID NO: 462 - protein, 9 aa, Homo sapiens
RPFHTRATV

SEQ ID NO: 463 - protein, 8 aa, Homo sapiens
TPKAGPTL

SEQ ID NO: 464 - protein, 9 aa, Homo sapiens
YPRPGTPAA

SEQ ID NO: 465 - protein, 9 aa, Homo sapiens
VPRPIFSQL

SEQ ID NO: 466 - protein, 9 aa, Homo sapiens
APYKSVTSL

SEQ ID NO: 467 - protein, 9 aa, Homo sapiens
KPFSSFTSM

SEQ ID NO: 468 - protein, 9 aa, Homo sapiens
SPMYGQAGL

SEQ ID NO: 469 - protein, 9 aa, Homo sapiens
YPENGVVQM

SEQ ID NO: 470 - protein, 9 aa, Homo sapiens
SPNSYFRVL

SEQ ID NO: 471 - protein, 10 aa, Homo sapiens
KPRPDVTNEL

SEQ ID NO: 472 - protein, 9 aa, Homo sapiens
NPRATDAQL

SEQ ID NO: 473 - protein, 9 aa, Homo sapiens
LPRALLSSL

SEQ ID NO: 474 - protein, 8 aa, Homo sapiens
LPRLLPAL

SEQ ID NO: 475 - protein, 9 aa, Homo sapiens
RPHKPGLYL

SEQ ID NO: 476 - protein, 9 aa, Homo sapiens
AEEEIMKKI

SEQ ID NO: 477 - protein, 9 aa, Homo sapiens
QENSYQSRL

SEQ ID NO: 478 - protein, 10 aa, Homo sapiens
SEIEQEIGSL

SEQ ID NO: 479 - protein, 9 aa, Homo sapiens
AEIQPQTQV

SEQ ID NO: 480 - protein, 10 aa, Homo sapiens
GEVSGLTKDF

SEQ ID NO: 481 - protein, 9 aa, Homo sapiens
RELQHEHSL

SEQ ID NO: 482 - protein, 9 aa, Homo sapiens
TEREWADEW

SEQ ID NO: 483 - protein, 10 aa, Homo sapiens
EENDQSTHKW

SEQ ID NO: 484 - protein, 9 aa, Homo sapiens
AEVGFVRFF

SEQ ID NO: 485 - protein, 11 aa, Homo sapiens
SEIEDSTKQVF

SEQ ID NO: 486 - protein, 9 aa, Homo sapiens
SEDDPILQI

SEQ ID NO: 487 - protein, 9 aa, Homo sapiens
AEDQLHHSF

SEQ ID NO: 488 - protein, 9 aa, Homo sapiens
TEFPIIKMY

SEQ ID NO: 489 - protein, 9 aa, Homo sapiens
SEIGKAVGF

SEQ ID NO: 490 - protein, 9 aa, Homo sapiens
SYVKVLHHL

SEQ ID NO: 491 - protein, 9 aa, Homo sapiens
KYLEKYYNL

SEQ ID NO: 492 - protein, 9 aa, Homo sapiens
NYEDHFPLL

SEQ ID NO: 493 - protein, 10 aa, Homo sapiens
TYKYVDINTF

SEQ ID NO: 494 - protein, 9 aa, Homo sapiens
RYLEKFYGL

SEQ ID NO: 495 - protein, 9 aa, Homo sapiens
SYNDALLTF

SEQ ID NO: 496 - protein, 10 aa, Homo sapiens
VFMKDGFFYF

SEQ ID NO: 497 - protein, 9 aa, Homo sapiens
NYPKSIHSF

SEQ ID NO: 498 - protein, 9 aa, Homo sapiens
EYIRALQQL

SEQ ID NO: 499 - protein, 9 aa, Homo sapiens
VYFVAPAKF

SEQ ID NO: 500 - protein, 10 aa, Homo sapiens
VWSDVTPLTF

SEQ ID NO: 501 - protein, 9 aa, Homo sapiens
GYIDNVTLI

SEQ ID NO: 502 - protein, 9 aa, Homo sapiens
SVHKITSTF

SEQ ID NO: 503 - protein, 12 aa, Homo sapiens
VHFEDTGKTLLF

SEQ ID NO: 504 - protein, 10 aa, Homo sapiens
VYEKNGYIYF

SEQ ID NO: 505 - protein, 9 aa, Homo sapiens
AYISGLDVF

SEQ ID NO: 506 - protein, 9 aa, Homo sapiens
RYVFPLPYL

SEQ ID NO: 507 - protein, 9 aa, Homo sapiens
VYIAELEKI

SEQ ID NO: 508 - protein, 9 aa, Homo sapiens
IYVTGGHLF

SEQ ID NO: 509 - protein, 9 aa, Homo sapiens
ALLEEEEGV

SEQ ID NO: 510 - protein, 9 aa, Homo sapiens
KVLEHVVRV

SEQ ID NO: 511 - protein, 11 aa, Homo sapiens
KIWEELSVLEV

SEQ ID NO: 512 - protein, 9 aa, Homo sapiens
VLGEEQEGV

SEQ ID NO: 513 - protein, 9 aa, Homo sapiens
KLVELEHTL

SEQ ID NO: 514 - protein, 11 aa, Homo sapiens
VQLDSIEDLEV

SEQ ID NO: 515 - protein, 9 aa, Homo sapiens
KIFEMLEGV

SEQ ID NO: 516 - protein, 9 aa, Homo sapiens
YTFSGDVQL

SEQ ID NO: 517 - protein, 11 aa, Homo sapiens
TLYNPERTITV

SEQ ID NO: 518 - protein, 11 aa, Homo sapiens
GLLEDERALQL

SEQ ID NO: 519 - protein, 9 aa, Homo sapiens
KIQEILTQV

SEQ ID NO: 520 - protein, 9 aa, Homo sapiens
KIQEMQHFL

SEQ ID NO: 521 - protein, 9 aa, Homo sapiens
FVYGEPREL

SEQ ID NO: 522 - protein, 9 aa, Homo sapiens
TLDEKVAEL

SEQ ID NO: 523 - protein, 9 aa, Homo sapiens
HLIAEIHTA

SEQ ID NO: 524 - protein, 9 aa, Homo sapiens
KVWSDVTPL

SEQ ID NO: 525 - protein, 9 aa, Homo sapiens
RLDDLKMTV

SEQ ID NO: 526 - protein, 9 aa, Homo sapiens
VLSPFILTL

SEQ ID NO: 527 - protein, 8 aa, Homo sapiens
LLDSVSRL

SEQ ID NO: 528 - protein, 9 aa, Homo sapiens
RLLDSVSRL

SEQ ID NO: 529 - protein, 9 aa, Homo sapiens
HPSAHDVIL

SEQ ID NO: 530 - protein, 10 aa, Homo sapiens
APAAWLRSAA

SEQ ID NO: 531 - protein, 9 aa, Homo sapiens
AEIEADRSY

SEQ ID NO: 532 - protein, 10 aa, Homo sapiens
ELAGIGILTV

SEQ ID NO: 533 - protein, 9 aa, Homo sapiens
YLLPAIVHI